European Patent Application EP 4 299 584 A1, published January 3, 2024. Title: mutant oestrogen receptor ligand binding domains. Applicant: Katholieke Universiteit Leuven VIB vzw. The sequence listing filed with the application follows.

SEQUENCE LISTING (58 sequences)

SEQ ID NO: 1 - protein, 22 aa, artificial sequence
  sequence fragment of mutant Human Estrogen Receptor Ligand Binding Domain
HLYSMKCKNVVPLYDLLLEMLD

SEQ ID NO: 2 - protein, 22 aa, artificial sequence
  sequence fragment of mutant Human Estrogen Receptor Ligand Binding Domain
HLYSMKCKNVVPLNDWILEMLD

SEQ ID NO: 3 - protein, 22 aa, artificial sequence
  sequence fragment of mutant Human Estrogen Receptor Ligand Binding Domain
HLYSMKCKNVVPLYDELLEMLD

SEQ ID NO: 4 - protein, 22 aa, artificial sequence
  sequence fragment of mutant Human Estrogen Receptor Ligand Binding Domain
HLYSMKCKNVVPLYDFLLEELD

SEQ ID NO: 5 - protein, 22 aa, artificial sequence
  sequence fragment of mutant Human Estrogen Receptor Ligand Binding Domain
HLYSMKCKNVVPLYDELLELLD

SEQ ID NO: 6 - protein, 22 aa, artificial sequence
  sequence fragment of mutant Human Estrogen Receptor Ligand Binding Domain
HVYSMKCKNVVPLYDELLELLD

SEQ ID NO: 7 - protein, 19 aa, artificial sequence
  sequence fragment of mutant Human Estrogen Receptor Ligand Binding Domain
HLYSMKCKNVVPLYDFTLE

SEQ ID NO: 8 - protein, 20 aa, artificial sequence
  sequence fragment of mutant Human Estrogen Receptor Ligand Binding Domain
HLYSMKCKNVVPLYDCNLET

SEQ ID NO: 9 - protein, 15 aa, artificial sequence
  sequence fragment of mutant Human Estrogen Receptor Ligand Binding Domain
YLYSMKCKNVVPLYD

SEQ ID NO: 10 - protein, 22 aa, artificial sequence
  sequence fragment of mutant Human Estrogen Receptor Ligand Binding Domain
YLYSMKCKNVVPLYDLLLEMLD

SEQ ID NO: 11 - protein, 20 aa, artificial sequence
  sequence fragment of mutant Human Estrogen Receptor Ligand Binding Domain
HLYSMKCKNVVPLYDLGLEV

SEQ ID NO: 12 - protein, 20 aa, artificial sequence
  sequence fragment of mutant Human Estrogen Receptor Ligand Binding Domain
HPYLMKCKNVVPLYDLALEY

SEQ ID NO: 13 - protein, 22 aa, artificial sequence
  sequence fragment of mutant Human Estrogen Receptor Ligand Binding Domain
HLYSMKCKNVVPLYDLLLEKLD

SEQ ID NO: 14 - protein, 22 aa, artificial sequence
  sequence fragment of mutant Human Estrogen Receptor Ligand Binding Domain
HKYLMKCKNVVPLYDLLLEAQD

SEQ ID NO: 15 - protein, 16 aa, artificial sequence
  sequence fragment of mutant Human Estrogen Receptor Ligand Binding Domain
HLYSMKCKNVVPLYDL

SEQ ID NO: 16 - protein, 22 aa, artificial sequence
  sequence fragment of mutant Human Estrogen Receptor Ligand Binding Domain
HPYSMKCKNVVPLYDWFLERLD

SEQ ID NO: 17 - protein, 19 aa, artificial sequence
  sequence fragment of mutant Human Estrogen Receptor Ligand Binding Domain
HLYSMKCKNVVPLYDDSLE

SEQ ID NO: 18 - protein, 5 aa, artificial sequence
  sequence fragment of mutant Human Estrogen Receptor Ligand Binding Domain
HLYSM

SEQ ID NO: 19 - protein, 21 aa, artificial sequence
  sequence fragment of mutant Human Estrogen Receptor Ligand Binding Domain
LYSMKCKNVVPLYDLLLEMLD

SEQ ID NO: 20 - protein, 7 aa, artificial sequence
  sequence fragment of mutant Human Estrogen Receptor Ligand Binding Domain
LLLEMLD

SEQ ID NO: 21 - protein, 5 aa, artificial sequence
  sequence fragment of mutant Human Estrogen Receptor Ligand Binding Domain
LYSMT

SEQ ID NO: 22 - protein, 8 aa, artificial sequence
  sequence fragment of mutant Human Estrogen Receptor Ligand Binding Domain
LYSMKCKN

SEQ ID NO: 23 - protein, 16 aa, artificial sequence
  sequence fragment of mutant Human Estrogen Receptor Ligand Binding Domain
CKNVVPLYDLLLEMLD

SEQ ID NO: 24 - protein, 4 aa, artificial sequence
  sequence fragment of mutant Human Estrogen Receptor Ligand Binding Domain
LYSM

SEQ ID NO: 25 - protein, 7 aa, artificial sequence
  sequence fragment of mutant Human Estrogen Receptor Ligand Binding Domain
LYSMKCK

SEQ ID NO: 26 - protein, 13 aa, artificial sequence
  sequence fragment of mutant Human Estrogen Receptor Ligand Binding Domain
LYSMKCKNVVPLY

SEQ ID NO: 27 - protein, 21 aa, artificial sequence
  sequence fragment of mutant Human Estrogen Receptor Ligand Binding Domain
LYSMKCKNVVPLNDWILEMLD

SEQ ID NO: 28 - protein, 7 aa, artificial sequence
  sequence fragment of mutant Human Estrogen Receptor Ligand Binding Domain
SDLEHED

SEQ ID NO: 29 - protein, 7 aa, artificial sequence
  sequence fragment of mutant Human Estrogen Receptor Ligand Binding Domain
FLLEMLD

SEQ ID NO: 30 - protein, 19 aa, artificial sequence
  sequence fragment of mutant Human Estrogen Receptor Ligand Binding Domain
LYSMKCKNVVPLYDLGLEV

SEQ ID NO: 31 - protein, 21 aa, artificial sequence
  sequence fragment of mutant Human Estrogen Receptor Ligand Binding Domain
LYSMKCKNVVPLYDELLEMLD

SEQ ID NO: 32 - protein, 21 aa, artificial sequence
  sequence fragment of mutant Human Estrogen Receptor Ligand Binding Domain
LYSMKCKNVVPLYDLILEMLD

SEQ ID NO: 33 - protein, 19 aa, artificial sequence
  sequence fragment of mutant Human Estrogen Receptor Ligand Binding Domain
LYSMKCKNVVPLYDFPLEM

SEQ ID NO: 34 - protein, 21 aa, artificial sequence
  sequence fragment of mutant Human Estrogen Receptor Ligand Binding Domain
LYSMKCKNVVPLYDLQLEMLD

SEQ ID NO: 35 - protein, 12 aa, artificial sequence
  sequence fragment of mutant Human Estrogen Receptor Ligand Binding Domain
PYLMKCKNVVPL

SEQ ID NO: 36 - protein, 12 aa, artificial sequence
  sequence fragment of mutant Human Estrogen Receptor Ligand Binding Domain
LYSMKCKNVVPL

SEQ ID NO: 37 - protein, 21 aa, artificial sequence
  sequence fragment of mutant Human Estrogen Receptor Ligand Binding Domain
LYSMKCKNVVPLYDLLLELLD

SEQ ID NO: 38 - protein, 15 aa, artificial sequence
  sequence fragment of mutant Human Estrogen Receptor Ligand Binding Domain
LYSMKCKNVVPLYDV

SEQ ID NO: 39 - protein, 6 aa, artificial sequence
  sequence fragment of mutant Human Estrogen Receptor Ligand Binding Domain
QKYYIT

SEQ ID NO: 40 - protein, 6 aa, artificial sequence
  sequence fragment of mutant Human Estrogen Receptor Ligand Binding Domain
QKYYIL

SEQ ID NO: 41 - protein, 5 aa, artificial sequence
  sequence fragment of mutant Human Estrogen Receptor Ligand Binding Domain
QKYYI

SEQ ID NO: 42 - protein, 17 aa, artificial sequence
  sequence fragment of mutant Human Estrogen Receptor Ligand Binding Domain
LEILMIGLVWRSMEHPG

SEQ ID NO: 43 - protein, 17 aa, artificial sequence
  sequence fragment of mutant Human Estrogen Receptor Ligand Binding Domain
MEILMIGLVWRSMEHPG

SEQ ID NO: 44 - protein, 17 aa, artificial sequence
  sequence fragment of mutant Human Estrogen Receptor Ligand Binding Domain
LEILLIGVVWRSMEHPG

SEQ ID NO: 45 - protein, 17 aa, artificial sequence
  sequence fragment of mutant Human Estrogen Receptor Ligand Binding Domain
FEILMIGLVWRSMEHPG

SEQ ID NO: 46 - protein, 17 aa, artificial sequence
  sequence fragment of mutant Human Estrogen Receptor Ligand Binding Domain
LEILMIGTVWRSMEHPG

SEQ ID NO: 47 - protein, 17 aa, artificial sequence
  sequence fragment of mutant Human Estrogen Receptor Ligand Binding Domain
LEILMIGLVWRSMEHPE

SEQ ID NO: 48 - protein, 17 aa, artificial sequence
  sequence fragment of mutant Human Estrogen Receptor Ligand Binding Domain
LEILMIGLVWRSMEHPH

SEQ ID NO: 49 - protein, 17 aa, artificial sequence
  sequence fragment of mutant Human Estrogen Receptor Ligand Binding Domain
LEILMIGLVWRSMEHPA

SEQ ID NO: 50 - protein, 17 aa, artificial sequence
  sequence fragment of mutant Human Estrogen Receptor Ligand Binding Domain
LEILMIGLVWRSMEHPS

SEQ ID NO: 51 - protein, 17 aa, artificial sequence
  sequence fragment of mutant Human Estrogen Receptor Ligand Binding Domain
LEILMIGLVWRSMEHPQ

SEQ ID NO: 52 - protein, 11 aa, artificial sequence
  sequence fragment of mutant Human Estrogen Receptor Ligand Binding Domain
PLYDFLLEELD

SEQ ID NO: 53 - protein, 11 aa, artificial sequence
  sequence fragment of mutant Human Estrogen Receptor Ligand Binding Domain
PLYDLLLEMLD

SEQ ID NO: 54 - protein, 10 aa, artificial sequence
  sequence fragment of mutant Human Estrogen Receptor Ligand Binding Domain
PLYDFLLELD

SEQ ID NO: 55 - protein, 595 aa, Homo sapiens [sequence omitted]

SEQ ID NO: 56 - protein, 21 aa, Artificial Sequence
  fragment of mutated estrogen receptor
CAWLEILMIGTVWRSMEHPGK

SEQ ID NO: 57 - protein, 25 aa, Artificial Sequence
  fragment of mutated estrogen receptor
KCKNVVPLYDFLLEELDAHRLHAPT

SEQ ID NO: 58 - protein, 173 aa, Artificial Sequence
  fragment of mutated estrogen receptor
CAWLEILMIGTVWRSMEHPGKLLFAPNLLLDRNQGKCVEGMVEIFDMLLATSSRFRMMNLQGEEFVCLKSIILLNSGVYTFLSSTLKSLEEKDHIHRVLDKITDTLIHLMAKAGLTLQQQHQRLAQLLLILSHIRHMSNKGMEHLYSMKCKNVVPLYDFLLEELDAHRLHAPT